European Patent Specification EP 3 597 664 B1, published November 26, 2025. Title: TEMPERATURE SHIFT FOR HIGH YIELD EXPRESSION OF POLYPEPTIDES IN YEAST AND OTHER TRANSFORMED CELLS. Applicant: ALDER BIOPHARMACEUTICALS, INC. The sequence listing filed with the application follows.

SEQUENCE LISTING (28 sequences)

SEQ ID NO: 1 - DNA, 1326 bp, Artificial
  Engineered antibody sequence
gaggtgcagcttgtggagtctgggggaggcttggtccagcctggggggtccctgagactctcctgtgcagtctctggaatcgacctcagtggctactacatgaactgggtccgtcaggctccagggaaggggctggagtgggtcggagtcattggtattaatggtgccacatactacgcgagctgggcgaaaggccgattcaccatctccagagacaattccaagaccacggtgtatcttcaaatgaacagcctgagagctgaggacactgctgtgtatttctgtgctagaggggacatctggggccaagggaccctcgtcaccgtctcgagcgcctccaccaagggcccatcggtcttccccctggcaccctcctccaagagcacctctgggggcacagcggccctgggctgcctggtcaaggactacttccccgaaccggtgacggtgtcgtggaactcaggcgccctgaccagcggcgtgcacaccttcccggctgtcctacagtcctcaggactctactccctcagcagcgtggtgaccgtgccctccagcagcttgggcacccagacctacatctgcaacgtgaatcacaagcccagcaacaccaaggtggacgcgagagttgagcccaaatcttgtgacaaaactcacacatgcccaccgtgcccagcacctgaactcctggggggaccgtcagtcttcctcttccccccaaaacccaaggacaccctcatgatctcccggacccctgaggtcacatgcgtggtggtggacgtgagccacgaagaccctgaggtcaagttcaactggtacgtggacggcgtggaggtgcataatgccaagacaaagccgcgggaggagcagtacgccagcacgtaccgtgtggtcagcgtcctcaccgtcctgcaccaggactggctgaatggcaaggagtacaagtgcaaggtctccaacaaagccctcccagcccccatcgagaaaaccatctccaaagccaaagggcagccccgagaaccacaggtgtacaccctgcccccatcccgggaggagatgaccaagaaccaggtcagcctgacctgcctggtcaaaggcttctatcccagcgacatcgccgtggagtgggagagcaatgggcagccggagaacaactacaagaccacgcctcccgtgctggactccgacggctccttcttcctctacagcaagctcaccgtggacaagagcaggtggcagcaggggaacgtcttctcatgctccgtgatgcatgaggctctgcacaaccactacacgcagaagagcctctccctgtctccgggtaaatga

SEQ ID NO: 2 - DNA, 660 bp, Artificial
  Engineered antibody sequence
caagtgctgacccagtctccatcctccctgtctgcatctgtaggagacagagtcaccatcaattgccaggccagtcagagtgtttatcataacacctacctggcctggtatcagcagaaaccagggaaagttcctaagcaactgatctatgatgcatccactctggcatctggggtcccatctcgtttcagtggcagtggatctgggacagatttcactctcaccatcagcagcctgcagcctgaagatgttgcaacttattactgtctgggcagttatgattgtactaatggtgattgttttgttttcggcggaggaaccaaggtggaaatcaaacgtacggtggctgcaccatctgtcttcatcttcccgccatctgatgagcagttgaaatctggaactgcctctgttgtgtgcctgctgaataacttctatcccagagaggccaaagtacagtggaaggtggataacgccctccaatcgggtaactcccaggagagtgtcacagagcaggacagcaaggacagcacctacagcctcagcagcaccctgacgctgagcaaagcagactacgagaaacacaaagtctacgcctgcgaagtcacccatcagggcctgagctcgcccgtcacaaagagcttcaacaggggagagtgttag

SEQ ID NO: 3 - DNA, 1350 bp, Artificial
  Engineered antibody sequence
gaggtgcagctggtggagtctgggggaggcttggtccagcctggggggtccctgagactctcctgtgcagcctctggattctccctcagtaactactacgtgacctgggtccgtcaggctccagggaaggggctggagtgggtcggcatcatctatggtagtgatgaaaccgcctacgctacctccgctataggccgattcaccatctccagagacaattccaagaacaccctgtatcttcaaatgaacagcctgagagctgaggacactgctgtgtattactgtgctagagatgatagtagtgactgggatgcaaagttcaacttgtggggccaagggaccctcgtcaccgtctcgagcgcctccaccaagggcccatcggtcttccccctggcaccctcctccaagagcacctctgggggcacagcggccctgggctgcctggtcaaggactacttccccgaaccggtgacggtgtcgtggaactcaggcgccctgaccagcggcgtgcacaccttcccggctgtcctacagtcctcaggactctactccctcagcagcgtggtgaccgtgccctccagcagcttgggcacccagacctacatctgcaacgtgaatcacaagcccagcaacaccaaggtggacaagagagttgagcccaaatcttgtgacaaaactcacacatgcccaccgtgcccagcacctgaactcctggggggaccgtcagtcttcctcttccccccaaaacccaaggacaccctcatgatctcccggacccctgaggtcacatgcgtggtggtggacgtgagccacgaagaccctgaggtcaagttcaactggtacgtggacggcgtggaggtgcataatgccaagacaaagccgcgggaggagcagtacgccagcacgtaccgtgtggtcagcgtcctcaccgtcctgcaccaggactggctgaatggcaaggagtacaagtgcaaggtctccaacaaagccctcccagcccccatcgagaaaaccatctccaaagccaaagggcagccccgagaaccacaggtgtacaccctgcccccatcccgggaggagatgaccaagaaccaggtcagcctgacctgcctggtcaaaggcttctatcccagcgacatcgccgtggagtgggagagcaatgggcagccggagaacaactacaagaccacgcctcccgtgctggactccgacggctccttcttcctctacagcaagctcaccgtggacaagagcaggtggcagcaggggaacgtcttctcatgctccgtgatgcatgaggctctgcacaaccactacacgcagaagagcctctccctgtctccgggtaaa

SEQ ID NO: 4 - DNA, 651 bp, Artificial
  Engineered antibody sequence
gctatccagatgacccagtctccttcctccctgtctgcatctgtaggagacagagtcaccatcacttgccaggccagtcagagcattaacaatgagttatcctggtatcagcagaaaccagggaaagcccctaagctcctgatctatagggcatccactctggcatctggggtcccatcaaggttcagcggcagtggatctgggacagacttcactctcaccatcagcagcctgcagcctgatgattttgcaacttattactgccaacagggttatagtctgaggaacattgataatgctttcggcggagggaccaaggtggaaatcaaacgtacggtggctgcaccatctgtcttcatcttcccgccatctgatgagcagttgaaatctggaactgcctctgttgtgtgcctgctgaataacttctatcccagagaggccaaagtacagtggaaggtggataacgccctccaatcgggtaactcccaggagagtgtcacagagcaggacagcaaggacagcacctacagcctcagcagcaccctgacgctgagcaaagcagactacgagaaacacaaagtctacgcctgcgaagtcacccatcagggcctgagctcgcccgtcacaaagagcttcaacaggggagagtgt

SEQ ID NO: 5 - protein, 18 aa, Artificial
  Secretion peptide
MRSLLILVLCFLPLAALG

SEQ ID NO: 6 - protein, 16 aa, Artificial
  Secretion peptide
MRLLLLLLLLPLAALG

SEQ ID NO: 7 - protein, 19 aa, Artificial
  Secretion peptide
MLLQAFLFLLAGFAAKISA

SEQ ID NO: 8 - protein, 35 aa, Artificial
  Secretion peptide
MRFPSIFTAVLFAASSALAAPVNTTTEEGVSLEKR

SEQ ID NO: 9 - protein, 22 aa, Artificial
  Secretion peptide
MRFPSIFTAVLFAASSALAAPV

SEQ ID NO: 10 - protein, 27 aa, Artificial
  Secretion peptide
MRFPSIFTAVLFAASSALAAPVSLEKR

SEQ ID NO: 11 - protein, 41 aa, Artificial
  Secretion peptide
MRFPSIFTAVLFAASSALAAPVNTTTEEGVSLEKREAEAEA

SEQ ID NO: 12 - protein, 85 aa, Artificial
  Secretion peptide
MRFPSIFTAVLFAASSALAAPVNTTTEDETAQIPAEAVIGYSDLEGDFDVAVLPFSNSTNNGLLFINTTIASIAAKEEGVSLEKR

SEQ ID NO: 13 - protein, 44 aa, Artificial
  Secretion peptide
MTKPTQVLVRSVSILFFITLLHLVVALNDVAGPAETAPVSLLPR

SEQ ID NO: 14 - protein, 22 aa, Artificial
  Secretion peptide
MFSPILSLEIILALATLQSVFA

SEQ ID NO: 15 - protein, 22 aa, Artificial
  Secretion peptide
MQTLLVSSLVVSLAAALPHYIR

SEQ ID NO: 16 - protein, 22 aa, Artificial
  Secretion peptide
MIFLKLIKSIVIGLGLVSAIQA

SEQ ID NO: 17 - protein, 24 aa, Artificial
  Secretion peptide
MKWVTFISLLFLFSSAYSRGVFRR

SEQ ID NO: 18 - protein, 18 aa, Artificial
  Secretion peptide
MKWVTFISLLFLFSSAYS

SEQ ID NO: 19 - protein, 24 aa, Artificial
  Secretion peptide
MALWMRLLPLLALLALWGPDPAAA

SEQ ID NO: 20 - protein, 24 aa, Artificial
  Secretion peptide
MKYTSYILAFQLCIVLGSLGCDLP

SEQ ID NO: 21 - protein, 26 aa, Artificial
  Secretion peptide
MAADSQTPWLLTFSLLCLLWPQEPGA

SEQ ID NO: 22 - protein, 27 aa, Artificial
  Secretion peptide
MKKNRMMMMIWSVGVVWMLLLVGGSYG

SEQ ID NO: 23 - protein, 18 aa, Artificial
  Secretion peptide
MQKLIIFALVVLCVGSEA

SEQ ID NO: 24 - protein, 18 aa, Artificial
  Secretion peptide
MKALIVLGLVLLSVTVQG

SEQ ID NO: 25 - protein, 20 aa, Artificial
  Secretion peptide
MVDGVMILPVLIMIALPSPS

SEQ ID NO: 26 - protein, 19 aa, Artificial
  Secretion peptide
MGAAAKLAFAVFLISCSSG

SEQ ID NO: 27 - protein, 31 aa, Artificial
  Secretion peptide
MLSLKPSWLTLAALMYAMLLVVVPFAKPVRA

SEQ ID NO: 28 - protein, 22 aa, Artificial
  Secretion peptide
MDMRVPAQLLGLLLLWLPGAKC